European Patent Application EP 4 317 172 A1, published February 7, 2024. Title: Immunoassay method for ICTP. Applicant: SEKISUI MEDICAL CO., LTD. The sequence listing filed with the application follows.

SEQUENCE LISTING (9 sequences)

SEQ ID NO: 1 - protein, 8 aa, Homo sapiens
GFDFSFLP

SEQ ID NO: 2 - protein, 7 aa, Homo sapiens
FDFSFLP

SEQ ID NO: 3 - protein, 9 aa, Homo sapiens
SAGFDFSFL

SEQ ID NO: 4 - protein, 7 aa, Homo sapiens
SAGFDFS

SEQ ID NO: 5 - protein, 25 aa, Artificial Sequence
  Peptide fragment
SAGFDFSFLFLPQPPQEKAHDGGRC

SEQ ID NO: 6 - protein, 15 aa, Artificial Sequence
  Peptide fragment
SAGFDFSFLPQPPQC

SEQ ID NO: 7 - protein, 15 aa, Artificial Sequence
  Peptide fragment
CSAGFDFSFLPQPPQ

SEQ ID NO: 8 - protein, 26 aa, Artificial Sequence
  Partial ICTP sequence
SAGFDFSFLPQPPQEKAHDGGRYYRA

SEQ ID NO: 9 - protein, 34 aa, Artificial Sequence
  Partial sequence in ICTP
PPGPPGPPSAGFDFSFLPQPPQEKAHDGGRYYRA